European Patent Specification EP 3 589 213 B1, published June 17, 2026. Title: NON-INVASIVE METHODS FOR SKIN SAMPLE COLLECTION AND ANALYSIS. Applicant: CHILDREN'S HOSPITAL MEDICAL CENTER ET AL. Application Not Yet Assigned. The sequence listing filed with the application follows.

SEQUENCE LISTING (2 sequences)

SEQ ID NO: 1 - DNA, 29 bp, Homo sapiens
ttcgtataggataaaaaatattgtattaa

SEQ ID NO: 2 - DNA, 29 bp, Homo sapiens
  misc_feature (3)..(3): methylated cytosine
ttcgtataggataaaaaatattgtattaa